European Patent Specification EP 3 899 031 B1, published July 30, 2025. Title: Target Enrichment. Applicant: New England Biolabs, Inc. The sequence listing filed with the application follows.

SEQUENCE LISTING (4 sequences)

SEQ ID NO: 1 - DNA, 81 bp, Artificial Sequence
  Synthetic construct
  misc_feature (33)..(44): n is a, c, g, or t
gatcggaagagcgtcgtgtagggaaagagtgtnnnnnnnnnnnnaggctatagtgtagatctcggtggtcgccgtatcatt

SEQ ID NO: 2 - DNA, 18 bp, Artificial Sequence
  Synthetic construct
aatgatacggcgaccacc

SEQ ID NO: 3 - DNA, 82 bp, Artificial Sequence
  Synthetic construct
  misc_feature (38)..(49): n is a, c, g, or t
aatgatacggcgaccaccgagatctacaccgaatacgnnnnnnnnnnnnacactctttccctacacgacgctcttccgatct

SEQ ID NO: 4 - DNA, 34 bp, Artificial Sequence
  Synthetic construct
agatcggaagagcacacgtctgaactccagtcac